European Patent Application EP 4 714 965 A1, published March 25, 2026. Title: 用于检测HIV抗体的重组抗原. Applicant: 菲鹏生物股份有限公司. Application WO. The sequence listing filed with the application follows.

SEQUENCE LISTING (11 sequences)

SEQ ID NO: 1 - protein, 161 aa, artificial sequence
LATAGSAMGAASLTLSAQSRTLLAGIVQQQQQLLDVVKRQQEMLRLTVWGTKNLQARVTAIEKYLKDQAQLNSWGCAFRQVCHTTVPWVNDSLSPDWKNMTWQEWEKQVRYLEANISQQLEQAQIQQEKNMYELQKLNSWDVFSNWFDLTSWIKYIQYGVY

SEQ ID NO: 2 - protein, 143 aa, artificial sequence
LATAGSAMGAASLTLSAQSRTLLAGIVQQQQQLLDVVKRQQEMLRLTVWGTKNLQARVTAIEKYLKDQAQLNSWGCAFRQVCHTTVPWVNDSLSPDWKNMTWQEWEKQVRYLEANISQQLEQAQIQQEKNMYELQKLNSWDVF

SEQ ID NO: 3 - protein, 129 aa, artificial sequence
LSAQSRTLLAGIVQQQQQLLDVVKRQQEMLRLTVWGTKNLQARVTAIEKYLKDQAQLNSWGCAFRQVCHTTVPWVNDSLSPDWKNMTWQEWEKQVRYLEANISQQLEQAQIQQEKNMYELQKLNSWDVF

SEQ ID NO: 4 - protein, 102 aa, artificial sequence
AIEKYLKDQAQLNSWGCAFRQVCHTTVPWVNDSLSPDWKNMTWQEWEKQVRYLEANISQQLEQAQIQQEKNMYELQKLNSWDVFSNWFDLTSWIKYIQYGVY

SEQ ID NO: 5 - protein, 141 aa, artificial sequence
TLTVQARQLLSGIVQQQSNLLRAIEAQQHLLQLTVWGIKQLQTRVLAIERYLQDQQLLGIWGCSGKLICTTAVPWNSSWSNKSQDEIWDNMTWMQWDKEISNYTYEIYTLIEESQNQQEKNEKDLLALDSWKNLWNWFDIT

SEQ ID NO: 6 - protein, 245 aa, artificial sequence
AIEKYLKDQAQLNSWGCAFRQVCHTTVPWVNDSLSPDWKNMTWQEWEKQVRYLEANISQQLEQAQIQQEKNMYELQKLNSWDVFSNWFDLTSWIKYIQYGVYRSTLTVQARQLLSGIVQQQSNLLRAIEAQQHLLQLTVWGIKQLQTRVLAIERYLQDQQLLGIWGCSGKLICTTAVPWNSSWSNKSQDEIWDNMTWMQWDKEISNYTYEIYTLIEESQNQQEKNEKDLLALDSWKNLWNWFDIT

SEQ ID NO: 7 - protein, 245 aa, artificial sequence
AIEKYLKDQAQLNSWGSAFRQVSHTTVPWVNDSLSPDWKNMTWQEWEKQVRYLEANISQQLEQAQIQQEKNMYELQKLNSWDVFSNWFDLTSWIKYIQYGVYRSTLTVQARQLLSGIVQQQSNLLRAIEAQQHLLQLTVWGIKQLQTRVLAIERYLQDQQLLGIWGSSGKLISTTAVPWNSSWSNKSQDEIWDNMTWMQWDKEISNYTYEIYTLIEESQNQQEKNEKDLLALDSWKNLWNWFDIT

SEQ ID NO: 8 - protein, 5 aa, artificial sequence
GGSGG

SEQ ID NO: 9 - protein, 18 aa, artificial sequence
KESGSVSSEQLAQFRSLD

SEQ ID NO: 10 - protein, 12 aa, artificial sequence
GSAGSAAGSGEF

SEQ ID NO: 11 - protein, 12 aa, artificial sequence
GGSGGEFGGSGG